European Patent Application EP 4 640 703 A2, published October 29, 2025. Title: ANTI-C1S ANTIBODIES AND METHODS OF USE. Applicant: CHUGAI SEIYAKU KABUSHIKI KAISHA. The sequence listing filed with the application follows.

SEQUENCE LISTING (88 sequences)

SEQ ID NO: 1 - protein, 673 aa, Homo sapiens
EPTMYGEILSPNYPQAYPSEVEKSWDIEVPEGYGIHLYFTHLDIELSENCAYDSVQIISGDTEEGRLCGQRSSNNPHSPIVEEFQVPYNKLQVIFKSDFSNEERFTGFAAYYVATDINECTDFVDVPCSHFCNNFIGGYFCSCPPEYFLHDDMKNCGVNCSGDVFTALIGEIASPNYPKPYPENSRCEYQIRLEKGFQVVVTLRREDFDVEAADSAGNCLDSLVFVAGDRQFGPYCGHGFPGPLNIETKSNALDIIFQTDLTGQKKGWKLRYHGDPMPCPKEDTPNSVWEPAKAKYVFRDVVQITCLDGFEVVEGRVGATSFYSTCQSNGKWSNSKLKCQPVDCGIPESIENGKVEDPESTLFGSVIRYTCEEPYYYMENGGGGEYHCAGNGSWVNEVLGPELPKCVPVCGVPREPFEEKQRIIGGSDADIKNFPWQVFFDNPWAGGALINEYWVLTAAHVVEGNREPTMYVGSTSVQTSRLAKSKMLTPEHVFIHPGWKLLEVPEGRTNFDNDIALVRLKDPVKMGPTVSPICLPGTSSDYNLMDGDLGLISGWGRTEKRDRAVRLKAARLPVAPLRKCKEVKVEKPTADAEAYVFTPNMICAGGEKGMDSCKGDSGGAFAVQDPNDKTKFYAAGLVSWGPQCGTYGLYTRVKNYVDWIMKTMQENSTPRED

SEQ ID NO: 2 - protein, 673 aa, Rattus norvegicus
EPTMYGEILSPNYPQAYPNEVVKTWDIEVPEGFGIHLYFTHLDMELSENCAYDSVQIISGGIEEERLCGQRTSKSPNSPTVEEFQFPYNRLQVVFTSDFSNEERFTGFAAYYSAVDVNECTDFTDVPCSHFCNNFIGGYFCSCPPEYFLHDDMRTCGVNCSGDVFTALIGEIASPNYPNPYPENSRCEYQIRLQEGFRLVLTIRREDFDVEPADSEGNCHDSLTFAAKNQQFGPYCGNGFPGPLTIKTQSNTLDIVFQTDLTGQNKGWKLRYHGDPIPCPKEISANSIWEPEKAKYVFKDVVKITCVDGFEVVEGNVGSTSFYSTCQSNGQWSNSRLECQPVDCGVPEPIENGKVEDPEDTVFGSVIHYTCEEPYYYMEQEEGGEYHCAANGSWVNDQLGVELPKCIPVCGVPTEPFKVQQRIFGGYSTKIQSFPWQVYFESPRGGGALIDEYWVLTAAHVVEGNSDPVMYVGSTLLKIERLRNAQRLITERVIIHPSWKQEDDLNTRTNFDNDIALVQLKDPVKMGPTVAPICLPETSSDYNPSEGDLGLISGWGRTENRTNVIQLRGAKLPITSLEKCQQVKVENPKARSNDYVFTDNMICAGEKGVDSCEGDSGGAFALPVPNVKDPKFYVAGLVSWGKKCGTYGIYTKVKNYVDWILKTMQENSGPKKD

SEQ ID NO: 3 - protein, 673 aa, Macaca fascicularis
EPTMYGEILSPNYPQAYPSEVEKSWDIEVPEGYGIHLYFTHLDIELSENCAYDSVQIMSGDIEEGRLCGQRTSNNPYSPIVEEFQVPYNKLQVIFKSDFSNEERFTGFAAYYVATDINECTDFVDAPCSHFCNNFIGGYFCSCPPEYFLHDDMKNCGVNCSGDVFTALIGEIASPNYPKPYPENSRCEYQIRLEKGFQVVVTVRREDFDVEPADSEGNCLDSLVFVAGDQQFGPYCGRGFPGPLNIETKSNVLDIIFQTDLTGQNKGWKLRYHGDPMPCPKEETPTSVWEPAKAKYVFRDVVRITCLDGFEVVEGRVGATSFHSTCQSNGKWSNSKLKCQPVDCGIPESIENGKVEDPESTLFGSVTRYTCEEPYYYMENGGNGQYHCASNGSWVNEALSPELPKCVPVCGVPREPFEGKQRIIGGSDADIKNFPWQVFFDNPWAGGALIDEYWVLTAAHVVEGNQEPTMYVGSTSVQTSRLAKSKMLTSERVFIHPGWKLLEVPEARTNFDNDIALVQLKDPVKMGPTVAPICLPGTSSDYNLMDGDLGLIAGWGRTEKRDRALRLKAARLPVAPLRKCREVKVENPKADAGAYVFTPNMICAGGEKGMDSCKGDSGGAFAVQDPNDKTKFYVAGLVSWGPQCGTYGLYTRVQNYVDWIKKTMQENSTPSKD

SEQ ID NO: 4 - protein, 30 aa, synthetic construct
  REGION 1..30: note = an artificially synthesized sequence
EVMLVESGGGLVKPGGSLRLSCAASGFTFS

SEQ ID NO: 5 - protein, 14 aa, synthetic construct
  REGION 1..14: note = an artificially synthesized sequence
WVRQAPGKGLEWVA

SEQ ID NO: 6 - protein, 32 aa, synthetic construct
  REGION 1..32: note = an artificially synthesized sequence
RFTISRDNSKDTLYLQMNSLRAEDTALYYCAR

SEQ ID NO: 7 - protein, 11 aa, synthetic construct
  REGION 1..11: note = an artificially synthesized sequence
WGQGTLVTVSS

SEQ ID NO: 8 - protein, 23 aa, synthetic construct
  REGION 1..23: note = an artificially synthesized sequence
QIVLTQSPATLSLSPGERATLSC

SEQ ID NO: 9 - protein, 15 aa, synthetic construct
  REGION 1..15: note = an artificially synthesized sequence
WYQQKPGKAPKLWIY

SEQ ID NO: 10 - protein, 32 aa, synthetic construct
  REGION 1..32: note = an artificially synthesized sequence
GVPSRFSGSGSGTDYTLTISSLQPEDFATYYC

SEQ ID NO: 11 - protein, 10 aa, synthetic construct
  REGION 1..10: note = an artificially synthesized sequence
FGQGTKLEIK

SEQ ID NO: 12 - protein, 30 aa, synthetic construct
  REGION 1..30: note = an artificially synthesized sequence
EVMLVESGGGLVKPGGSLRLSCAASGFEFE

SEQ ID NO: 13 - protein, 118 aa, synthetic construct
  REGION 1..118: note = an artificially synthesized sequence
EVMLVESGGGLVKPGGSLRLSCAASGFTFSNYAMSWVRQAPGKGLEWVATISSGGSHTYYLDSVKGRFTISRDNSKDTLYLQMNSLRAEDTALYYCARLFTGYAMDYWGQGTLVTVSS

SEQ ID NO: 14 - protein, 109 aa, synthetic construct
  REGION 1..109: note = an artificially synthesized sequence
QIVLTQSPATLSLSPGERATLSCTASSSVSSSYLHWYQQKPGKAPKLWIYSTSNLASGVPSRFSGSGSGTDYTLTISSLQPEDFATYYCHQYYRLPPITFGQGTKLEIK

SEQ ID NO: 15 - protein, 327 aa, synthetic construct
  REGION 1..327: note = an artificially synthesized sequence
ASTKGPSVFPLAPCSRSTSESTAALGCLVKDYFPEPVTVSWNSGALTSGVHTFPAVLQSSGLYSLSSVVTVPSSSLGTKTYTCNVDHKPSNTKVDKRVESKYGPPCPPCPAPEFLGGPSVFLFPPKPKDTLMISRTPEVTCVVVDVSQEDPEVQFNWYVDGVEVHNAKTKPREEQFNSTYRVVSVLTVLHQDWLNGKEYKCKVSNKGLPSSIEKTISKAKGQPREPQVYTLPPSQEEMTKNQVSLTCLVKGFYPSDIAVEWESNGQPENNYKTTPPVLDSDGSFFLYSKLTVDKSRWQEGNVFSCSVMHEALHNHYTQKSLSLSLGK

SEQ ID NO: 16 - protein, 107 aa, synthetic construct [sequence omitted]

SEQ ID NO: 17 - protein, 118 aa, synthetic construct
  REGION 1..118: note = an artificially synthesized sequence
EVMLVESGGGLVKPGGSLRLSCAASGFTFSNYAMSWVRQAPGKGLEWVATISSGGSHTYYLDSVKGRFTISRDNSKDTLYLQMNSLRAEDTALYYCARLFTGHAMDYWGQGTLVTVSS

SEQ ID NO: 18 - protein, 109 aa, synthetic construct
  REGION 1..109: note = an artificially synthesized sequence
QIVLTQSPATLSLSPGERATLSCTASSSVSSSYLHWYQQKPGKAPKLWIYSTSNLASGVPSRFSGSGSGTDYTLTISSLQPEDFATYYCHQYYRLHPITFGQGTKLEIK

SEQ ID NO: 19 - protein, 118 aa, synthetic construct
  REGION 1..118: note = an artificially synthesized sequence
EVMLVESGGGLVKPGGSLRLSCAASGFTFSNYAMSWVRQAPGKGLEWVATISSGGSHTYELDSVDGRFTISRDNSKDTLYLQMNSLRAEDTALYYCARLFTKHAMDYWGQGTLVTVSS

SEQ ID NO: 20 - protein, 109 aa, synthetic construct
  REGION 1..109: note = an artificially synthesized sequence
QIVLTQSPATLSLSPGERATLSCTASSEVSESYLHWYQQKPGKAPKLWIYSTSNLASGVPSRFSGSGSGTDYTLTISSLQPEDFATYYCHQYYRLHPITFGQGTKLEIK

SEQ ID NO: 21 - protein, 109 aa, synthetic construct
  REGION 1..109: note = an artificially synthesized sequence
QIVLTQSPATLSLSPGERATLSCTASSEVSSSYLHWYQQKPGKAPKLWIYSTSNLASGVPSRFSGSGSGTDYTLTISSLQPEDFATYYCHQYYRLHPITFGQGTKLEIK

SEQ ID NO: 22 - protein, 118 aa, synthetic construct
  REGION 1..118: note = an artificially synthesized sequence
EVMLVESGGGLVKPGGSLRLSCAASGFEFENYAMSWVRQAPGKGLEWVATISSGGSHTYELDSVDGRFTISRDNSKDTLYLQMNSLRAEDTALYYCARLFTKHAMDYWGQGTLVTVSS

SEQ ID NO: 23 - protein, 5 aa, synthetic construct
  REGION 1..5: note = an artificially synthesized sequence
NYAMS

SEQ ID NO: 24 - protein, 17 aa, synthetic construct
  REGION 1..17: note = an artificially synthesized sequence
TISSGGSHTYYLDSVKG

SEQ ID NO: 25 - protein, 9 aa, synthetic construct
  REGION 1..9: note = an artificially synthesized sequence
LFTGYAMDY

SEQ ID NO: 26 - protein, 12 aa, synthetic construct
  REGION 1..12: note = an artificially synthesized sequence
TASSSVSSSYLH

SEQ ID NO: 27 - protein, 7 aa, synthetic construct
  REGION 1..7: note = an artificially synthesized sequence
STSNLAS

SEQ ID NO: 28 - protein, 10 aa, synthetic construct
  REGION 1..10: note = an artificially synthesized sequence
HQYYRLPPIT

SEQ ID NO: 29 - protein, 12 aa, synthetic construct
  REGION 1..12: note = an artificially synthesized sequence
GFNIKDDYIHWV

SEQ ID NO: 30 - protein, 10 aa, synthetic construct
  REGION 1..10: note = an artificially synthesized sequence
IDPADDHTKY

SEQ ID NO: 31 - protein, 12 aa, synthetic construct
  REGION 1..12: note = an artificially synthesized sequence
AIYGSGWAWFPY

SEQ ID NO: 32 - protein, 12 aa, synthetic construct
  REGION 1..12: note = an artificially synthesized sequence
QSVDYDGDSYMN

SEQ ID NO: 33 - protein, 10 aa, synthetic construct
  REGION 1..10: note = an artificially synthesized sequence
AASNLESGIP

SEQ ID NO: 34 - protein, 9 aa, synthetic construct
  REGION 1..9: note = an artificially synthesized sequence
QQSNEDPWT

SEQ ID NO: 35 - protein, 118 aa, synthetic construct; identical to SEQ ID NO: 13
  REGION 1..118: note = an artificially synthesized sequence

SEQ ID NO: 36 - protein, 118 aa, synthetic construct
  REGION 1..118: note = an artificially synthesized sequence
EVQLVESGGGLVKPGGSLRLSCAASGFTFSNYAMSWVRQAPGKGLEWVATISSGGSHTYYLDSVKGRFTISRDNSKNTLYLQMNSLRAEDTALYYCARLFTGYAMDYWGQGTLVTVSS

SEQ ID NO: 37 - protein, 109 aa, synthetic construct; identical to SEQ ID NO: 14
  REGION 1..109: note = an artificially synthesized sequence

SEQ ID NO: 38 - protein, 109 aa, synthetic construct
  REGION 1..109: note = an artificially synthesized sequence
QIVLTQSPATLSLSPGERATMSCTASSSVSSSYLHWYQQKPGKAPKLWIYSTSNLASGVPSRFSGSGSGTDYTLTISSLQPEDFATYYCHQYYRLPPITFGQGTKLEIK

SEQ ID NO: 39 - protein, 5 aa, synthetic construct
  REGION 1..5: note = an artificially synthesized sequence
NYAMS

SEQ ID NO: 40 - protein, 17 aa, synthetic construct
  REGION 1..17: note = an artificially synthesized sequence
TISSGGSHTYELDSVDG

SEQ ID NO: 41 - protein, 9 aa, synthetic construct
  REGION 1..9: note = an artificially synthesized sequence
LFTKHAMDY

SEQ ID NO: 42 - protein, 12 aa, synthetic construct
  REGION 1..12: note = an artificially synthesized sequence
TASSEVSESYLH

SEQ ID NO: 43 - protein, 7 aa, synthetic construct
  REGION 1..7: note = an artificially synthesized sequence
STSNLAS

SEQ ID NO: 44 - protein, 10 aa, synthetic construct
  REGION 1..10: note = an artificially synthesized sequence
HQYYRLHPIT

SEQ ID NO: 45 - protein, 12 aa, synthetic construct
  REGION 1..12: note = an artificially synthesized sequence
TASSEVSSSYLH

SEQ ID NO: 46 - protein, 115 aa, synthetic construct
  REGION 1..115: note = an artificially synthesized sequence
QSVEESGGRLVTPGTPLTLTCTVSGFSLTKYTVSWVRQAPGKGLEWIGIINTGGSAYYATWAKGRFTFSKTSTTVDLQITSPTTEDTATYFCARGNGDTDYTNLWGPGTLVTVSS

SEQ ID NO: 47 - protein, 117 aa, synthetic construct
  REGION 1..117: note = an artificially synthesized sequence
QSVEESGGRLVTPGTPLTLTCTVSGFSLSSYPMGWVRQVPGEGLEWIGTISAGGSTYYPSWAKGRFTISRTSTTVDLKMTSLTTEDTATYFCARGYPYTDGTYMTLWGPGTLVTVSS

SEQ ID NO: 48 - protein, 118 aa, synthetic construct
  REGION 1..118: note = an artificially synthesized sequence
QSVEESGGRLVTPGTPLTLTCTVSGIDLNNYPMGWVRQAPGKGLEYIGIISSSGGTSYASWAKGRFTISKTSSTTVDLKMTSLTTEDTATYFCARGYPYRDITYFNLWGPGTLVTVSS

SEQ ID NO: 49 - protein, 113 aa, synthetic construct
  REGION 1..113: note = an artificially synthesized sequence
QSLEESGGRLVTPGTPLTLTCTVSGFSLSSYTMIWVRQAPGKGLEWIGVVGGSGITYYASWAKGRFTISKTSTTVDLQITSPTTEDTATYFCARDTSVAGDLWGPGTLVTVSS

SEQ ID NO: 50 - protein, 117 aa, synthetic construct
  REGION 1..117: note = an artificially synthesized sequence
QSVEESGGRLVTPGGSLTLTCTVSGFSLSRNAINWVRQAPGKGLEWIGGVSGGATTYYASWANGRFTISKTSTTVDLKMTGLTAADTATYFCARGAGSNIDGPFNLWGPGTLVTVSS

SEQ ID NO: 51 - protein, 106 aa, synthetic construct
  REGION 1..106: note = an artificially synthesized sequence
QVLTQTPSSVSEPVGGTVTINCQASENIYSALAWYQQKPGQPPKLLIYGASNLESGVPSRFKGSGSGTQFTLTISDLECADAATYYCQQYYFTSSTFGGGTKVEIK

SEQ ID NO: 52 - protein, 108 aa, synthetic construct
  REGION 1..108: note = an artificially synthesized sequence
AFELTQTPSSVEAAVGGTVTIKCQASENIYSLLAWYQQKPGQPPKLLIYGASTLASGVSSRFSGSGYGTEFTLTISDLECADAATYYCQSYYDSSTTTFGGGTKVEIK

SEQ ID NO: 53 - protein, 110 aa, synthetic construct
  REGION 1..110: note = an artificially synthesized sequence
DPVLTQTPSPVSAPVGGSVTIKCQASQNIYSYLSWYQHKPGQPPKLLIYGASTLTNGVSSRFTGSGYGTEFTLTISDLECEDAATYYCQNYYSGGSADTTFGGGTKVEIK

SEQ ID NO: 54 - protein, 110 aa, synthetic construct
  REGION 1..110: note = an artificially synthesized sequence
AYDMTQTPASVEVAVGGTVTIKCQASQSIGVSLAWYQQKPGQRPKLLIYKASNLASGVPSRFKGSGSGTQFTLTISGVECADAATYYCQQDYTYSDVTNIFGGGTKVEIK

SEQ ID NO: 55 - protein, 108 aa, synthetic construct
  REGION 1..108: note = an artificially synthesized sequence
AFEMTQTPSSVSAPVGGTVTIKCQASQNIYSYLSWYQQKPGHPPKLLIYGASTLASGVPSRFKGSGYGTEFTLTISDLECADPATYYCQQYYATTSVDFGGGTKVEIK

SEQ ID NO: 56 - protein, 5 aa, synthetic construct
  REGION 1..5: note = an artificially synthesized sequence
KYTVS

SEQ ID NO: 57 - protein, 16 aa, synthetic construct
  REGION 1..16: note = an artificially synthesized sequence
IINTGGSAYYATWAKG

SEQ ID NO: 58 - protein, 10 aa, synthetic construct
  REGION 1..10: note = an artificially synthesized sequence
GNGDTDYTNL

SEQ ID NO: 59 - protein, 5 aa, synthetic construct
  REGION 1..5: note = an artificially synthesized sequence
SYPMG

SEQ ID NO: 60 - protein, 16 aa, synthetic construct
  REGION 1..16: note = an artificially synthesized sequence
TISAGGSTYYPSWAKG

SEQ ID NO: 61 - protein, 12 aa, synthetic construct
  REGION 1..12: note = an artificially synthesized sequence
GYPYTDGTYMTL

SEQ ID NO: 62 - protein, 5 aa, synthetic construct
  REGION 1..5: note = an artificially synthesized sequence
NYPMG

SEQ ID NO: 63 - protein, 16 aa, synthetic construct
  REGION 1..16: note = an artificially synthesized sequence
IISSSGGTSYASWAKG

SEQ ID NO: 64 - protein, 12 aa, synthetic construct
  REGION 1..12: note = an artificially synthesized sequence
GYPYRDITYFNL

SEQ ID NO: 65 - protein, 5 aa, synthetic construct
  REGION 1..5: note = an artificially synthesized sequence
SYTMI

SEQ ID NO: 66 - protein, 16 aa, synthetic construct
  REGION 1..16: note = an artificially synthesized sequence
VVGGSGITYYASWAKG

SEQ ID NO: 67 - protein, 8 aa, synthetic construct
  REGION 1..8: note = an artificially synthesized sequence
DTSVAGDL

SEQ ID NO: 68 - protein, 5 aa, synthetic construct
  REGION 1..5: note = an artificially synthesized sequence
RNAIN

SEQ ID NO: 69 - protein, 16 aa, synthetic construct
  REGION 1..16: note = an artificially synthesized sequence
GVSGGATTYYASWANG

SEQ ID NO: 70 - protein, 12 aa, synthetic construct
  REGION 1..12: note = an artificially synthesized sequence
GAGSNIDGPFNL

SEQ ID NO: 71 - protein, 11 aa, synthetic construct
  REGION 1..11: note = an artificially synthesized sequence
QASENIYSALA

SEQ ID NO: 72 - protein, 7 aa, synthetic construct
  REGION 1..7: note = an artificially synthesized sequence
GASNLES

SEQ ID NO: 73 - protein, 9 aa, synthetic construct
  REGION 1..9: note = an artificially synthesized sequence
QQYYFTSST

SEQ ID NO: 74 - protein, 11 aa, synthetic construct
  REGION 1..11: note = an artificially synthesized sequence
QASENIYSLLA

SEQ ID NO: 75 - protein, 7 aa, synthetic construct
  REGION 1..7: note = an artificially synthesized sequence
GASTLAS

SEQ ID NO: 76 - protein, 10 aa, synthetic construct
  REGION 1..10: note = an artificially synthesized sequence
QSYYDSSTTT

SEQ ID NO: 77 - protein, 11 aa, synthetic construct
  REGION 1..11: note = an artificially synthesized sequence
QASQNIYSYLS

SEQ ID NO: 78 - protein, 7 aa, synthetic construct
  REGION 1..7: note = an artificially synthesized sequence
GASTLTN

SEQ ID NO: 79 - protein, 12 aa, synthetic construct
  REGION 1..12: note = an artificially synthesized sequence
QNYYSGGSADTT

SEQ ID NO: 80 - protein, 11 aa, synthetic construct
  REGION 1..11: note = an artificially synthesized sequence
QASQSIGVSLA

SEQ ID NO: 81 - protein, 7 aa, synthetic construct
  REGION 1..7: note = an artificially synthesized sequence
KASNLAS

SEQ ID NO: 82 - protein, 12 aa, synthetic construct
  REGION 1..12: note = an artificially synthesized sequence
QQDYTYSDVTNI

SEQ ID NO: 83 - protein, 11 aa, synthetic construct
  REGION 1..11: note = an artificially synthesized sequence
QASQNIYSYLS

SEQ ID NO: 84 - protein, 7 aa, synthetic construct
  REGION 1..7: note = an artificially synthesized sequence
GASTLAS

SEQ ID NO: 85 - protein, 10 aa, synthetic construct
  REGION 1..10: note = an artificially synthesized sequence
QQYYATTSVD

SEQ ID NO: 86 - protein, 328 aa, synthetic construct
  REGION 1..328: note = an artificially synthesized sequence
ASTKGPSVFPLAPSSKSTSGGTAALGCLVKDYFPEPVTVSWNSGALTSGVHTFPAVLQSSGLYSLSSVVTVPSSSLGTQTYICNVNHKPSNTKVDKKVEPKSCDKTHTCPPCPAPELLGGPSVFLFPPKPKDTLMISRTPEVTCVVVDVSHEDPEVKFNWYVDGVEVHNAKTKPREEQYNSTYRVVSVLTVLHQDWLNGKEYKCEVSNKALPAPIEKTISKAKGQPREPQVYTLPPSREEMTKNQVSLTCLVKGFYPSDIAVEWESNGQPENNYKTTPPVLDSDGSFFLYSKLTVDKSRWQQGNVFSCSVMHEALHNHYTQKSLSLSP

SEQ ID NO: 87 - protein, 328 aa, synthetic construct
  REGION 1..328: note = an artificially synthesized sequence
ASTKGPSVFPLAPSSKSTSGGTAALGCLVKDYFPEPVTVSWNSGALTSGVHTFPAVLQSSGLYSLSSVVTVPSSSLGTQTYICNVNHKPSNTKVDKKVEPKSCDKTHTCPPCPAPELRRGPSVFLFPPKPKDTLMISRTPEVTCVVVDVSHEDPEVKFNWYVDGVEVHNAKTKPREEQYNSTYRVVSVLTVLHQDWLNGKEYKCKVSNKGLPSSIEKTISKAKGQPREPQVYTLPPSREEMTKNQVSLTCLVKGFYPSDIAVEWESNGQPENNYKTTPPVLDSDGSFFLYSKLTVDKSRWQQGNVFSCSVMHEALHNHYTQKSLSLSP

SEQ ID NO: 88 - protein, 107 aa, synthetic construct
  REGION 1..107: note = an artificially synthesized sequence
RTVAAPSVFIFPPSDEQLKSGTASVVCLLNNFYPREAKVQWKVDNALQSGNSQESVTEQDSKDCTYSLSSTLTLSKADYEKHKVYACEVTHQGLSSPVTKSFNRGEC